European Patent Application EP 4 553 169 A1, published May 14, 2025. Title: METHODS AND REAGENTS FOR THE MULTIPLEXED DETECTION OF NUCLEIC ACIDS. Applicant: PAPERDROP DIAGNOSTICS, S.L. Application EP. The sequence listing filed with the application follows.

SEQUENCE LISTING (24 sequences)

SEQ ID NO: 1 - DNA, 14 bp, synthetic construct
  source 1..14: mol_type = other DNA
gttttcccagtcac

SEQ ID NO: 2 - DNA, 14 bp, synthetic construct
  source 1..14: mol_type = other DNA
ttggtcgtggtggt

SEQ ID NO: 3 - DNA, 14 bp, synthetic construct
  source 1..14: mol_type = other DNA
catctttattagct

SEQ ID NO: 4 - DNA, 14 bp, synthetic construct
  source 1..14: mol_type = other DNA
gtttagcacatcag

SEQ ID NO: 5 - DNA, 14 bp, synthetic construct
  source 1..14: mol_type = other DNA
aacgctcacccatg

SEQ ID NO: 6 - DNA, 14 bp, synthetic construct
  source 1..14: mol_type = other DNA
cggagttgaggtga

SEQ ID NO: 7 - DNA, 14 bp, synthetic construct
  source 1..14: mol_type = other DNA
tctagtagtggatc

SEQ ID NO: 8 - DNA, 14 bp, synthetic construct
  source 1..14: mol_type = other DNA
ctatggtgaacgaa

SEQ ID NO: 9 - DNA, 32 bp, synthetic construct
  source 1..32: mol_type = other DNA
gtcgtgactgggaaaacttttttttttttttt

SEQ ID NO: 10 - DNA, 17 bp, synthetic construct
  source 1..17: mol_type = other DNA
gttttcccagtcacgac

SEQ ID NO: 11 - DNA, 29 bp, synthetic construct
  source 1..29: mol_type = other DNA
accaccacgaccaattttttttttttttt

SEQ ID NO: 12 - DNA, 19 bp, synthetic construct
  source 1..19: mol_type = other DNA
ttggtcgtggtggtggttt

SEQ ID NO: 13 - DNA, 29 bp, synthetic construct
  source 1..29: mol_type = other DNA
agctaataaagatgttttttttttttttt

SEQ ID NO: 14 - DNA, 29 bp, synthetic construct
  source 1..29: mol_type = other DNA
gcacgtattgtgcattttttttttttttt

SEQ ID NO: 15 - DNA, 14 bp, synthetic construct
  source 1..14: mol_type = other DNA
tgcacaatacgtgc

SEQ ID NO: 16 - DNA, 29 bp, synthetic construct
  source 1..29: mol_type = other DNA
ctgatgtgctaaacttttttttttttttt

SEQ ID NO: 17 - DNA, 31 bp, synthetic construct
  source 1..31: mol_type = other DNA
gtgactgggaaaacggttttttttttttttt

SEQ ID NO: 18 - DNA, 31 bp, synthetic construct
  source 1..31: mol_type = other DNA
accaccacgaccaaccttttttttttttttt

SEQ ID NO: 19 - DNA, 31 bp, synthetic construct
  source 1..31: mol_type = other DNA
agctaataaagatgagttttttttttttttt

SEQ ID NO: 20 - DNA, 31 bp, synthetic construct
  source 1..31: mol_type = other DNA
ctgatgtgctaaactcttttttttttttttt

SEQ ID NO: 21 - DNA, 31 bp, synthetic construct
  source 1..31: mol_type = other DNA
catgggtgagcgttctttttttttttttttt

SEQ ID NO: 22 - DNA, 31 bp, synthetic construct
  source 1..31: mol_type = other DNA
tcacctcaactccgaattttttttttttttt

SEQ ID NO: 23 - DNA, 31 bp, synthetic construct
  source 1..31: mol_type = other DNA
gatccactactagacgttttttttttttttt

SEQ ID NO: 24 - DNA, 31 bp, synthetic construct
  source 1..31: mol_type = other DNA
ttcgttcaccatagccttttttttttttttt